European Patent Specification EP 3 645 573 B1, published October 16, 2024. Title: NOVEL T CELL RECEPTORS AND IMMUNE THERAPY USING THE SAME. Applicant: Immatics Biotechnologies GmbH. The sequence listing filed with the application follows.

SEQUENCE LISTING (159 sequences)

SEQ ID NO: 1 - protein, 6 aa, Homo sapiens
DSSSTY

SEQ ID NO: 2 - protein, 3 aa, Homo sapiens
IFS

SEQ ID NO: 3 - protein, 13 aa, Homo sapiens
CAEIDNQGGKLIF

SEQ ID NO: 4 - protein, 132 aa, Homo sapiens
MKTFAGFSFLFLWLQLDCMSRGEDVEQSLFLSVREGDSSVINCTYTDSSSTYLYWYKQEPGAGLQLLTYIFSNMDMKQDQRLTVLLNKKDKHLSLRIADTQTGDSAIYFCAEIDNQGGKLIFGQGTELSVKP

SEQ ID NO: 5 - protein, 141 aa, Homo sapiens
NIQNPDPAVYQLRDSKSSDKSVCLFTDFDSQTNVSQSKDSDVYITDKTVLDMRSMDFKSNSAVAWSNKSDFACANAFNNSIIPEDTFFPSPESSCDVKLVEKSFETDTNLNFQNLSVIGFRILLLKVAGFNLLMTLRLWSS

SEQ ID NO: 6 - protein, 273 aa, Homo sapiens
MKTFAGFSFLFLWLQLDCMSRGEDVEQSLFLSVREGDSSVINCTYTDSSSTYLYWYKQEPGAGLQLLTYIFSNMDMKQDQRLTVLLNKKDKHLSLRIADTQTGDSAIYFCAEIDNQGGKLIFGQGTELSVKPNIQNPDPAVYQLRDSKSSDKSVCLFTDFDSQTNVSQSKDSDVYITDKTVLDMRSMDFKSNSAVAWSNKSDFACANAFNNSIIPEDTFFPSPESSCDVKLVEKSFETDTNLNFQNLSVIGFRILLLKVAGFNLLMTLRLWSS

SEQ ID NO: 7 - protein, 5 aa, Homo sapiens
SGHDT

SEQ ID NO: 8 - protein, 6 aa, Homo sapiens
YYEEEE

SEQ ID NO: 9 - protein, 12 aa, Homo sapiens
CASSQLNTEAFF

SEQ ID NO: 10 - protein, 130 aa, Homo sapiens
MGPGLLCWALLCLLGAGLVDAGVTQSPTHLIKTRGQQVTLRCSPKSGHDTVSWYQQALGQGPQFIFQYYEEEERQRGNFPDRFSGHQFPNYSSELNVNALLLGDSALYLCASSQLNTEAFFGQGTRLTVV

SEQ ID NO: 11 - protein, 177 aa, Homo sapiens
EDLNKVFPPEVAVFEPSEAEISHTQKATLVCLATGFFPDHVELSWWVNGKEVHSGVSTDPQPLKEQPALNDSRYCLSSRLRVSATFWQNPRNHFRCQVQFYGLSENDEWTQDRAKPVTQIVSAEAWGRADCGFTSVSYQQGVLSATILYEILLGKATLYAVLVSALVLMAMVKRKDF

SEQ ID NO: 12 - protein, 307 aa, Homo sapiens
MGPGLLCWALLCLLGAGLVDAGVTQSPTHLIKTRGQQVTLRCSPKSGHDTVSWYQQALGQGPQFIFQYYEEEERQRGNFPDRFSGHQFPNYSSELNVNALLLGDSALYLCASSQLNTEAFFGQGTRLTVVEDLNKVFPPEVAVFEPSEAEISHTQKATLVCLATGFFPDHVELSWWVNGKEVHSGVSTDPQPLKEQPALNDSRYCLSSRLRVSATFWQNPRNHFRCQVQFYGLSENDEWTQDRAKPVTQIVSAEAWGRADCGFTSVSYQQGVLSATILYEILLGKATLYAVLVSALVLMAMVKRKDF

SEQ ID NO: 13 - protein, 6 aa, Homo sapiens
DRGSQS

SEQ ID NO: 14 - protein, 2 aa, Homo sapiens
IY

SEQ ID NO: 15 - protein, 10 aa, Homo sapiens
CAVNNARLMF

SEQ ID NO: 16 - protein, 129 aa, Homo sapiens
MKSLRVLLVILWLQLSWVWSQQKEVEQNSGPLSVPEGAIASLNCTYSDRGSQSFFWYRQYSGKSPELIMFIYSNGDKEDGRFTAQLNKASQYVSLLIRDSQPSDSATYLCAVNNARLMFGDGTQLVVKP

SEQ ID NO: 17 - protein, 141 aa, Homo sapiens; identical to SEQ ID NO: 5

SEQ ID NO: 18 - protein, 270 aa, Homo sapiens
MKSLRVLLVILWLQLSWVWSQQKEVEQNSGPLSVPEGAIASLNCTYSDRGSQSFFWYRQYSGKSPELIMFIYSNGDKEDGRFTAQLNKASQYVSLLIRDSQPSDSATYLCAVNNARLMFGDGTQLVVKPNIQNPDPAVYQLRDSKSSDKSVCLFTDFDSQTNVSQSKDSDVYITDKTVLDMRSMDFKSNSAVAWSNKSDFACANAFNNSIIPEDTFFPSPESSCDVKLVEKSFETDTNLNFQNLSVIGFRILLLKVAGFNLLMTLRLWSS

SEQ ID NO: 19 - protein, 5 aa, Homo sapiens
SNHLY

SEQ ID NO: 20 - protein, 6 aa, Homo sapiens
FYNNEI

SEQ ID NO: 21 - protein, 13 aa, Homo sapiens
CASSGQGANEQYF

SEQ ID NO: 22 - protein, 132 aa, Homo sapiens
MDTWLVCWAIFSLLKAGLTEPEVTQTPSHQVTQMGQEVILRCVPISNHLYFYWYRQILGQKVEFLVSFYNNEISEKSEIFDDQFSVERPDGSNFTLKIRSTKLEDSAMYFCASSGQGANEQYFGPGTRLTVT

SEQ ID NO: 23 - protein, 179 aa, Homo sapiens
EDLKNVFPPEVAVFEPSEAEISHTQKATLVCLATGFYPDHVELSWWVNGKEVHSGVSTDPQPLKEQPALNDSRYCLSSRLRVSATFWQNPRNHFRCQVQFYGLSENDEWTQDRAKPVTQIVSAEAWGRADCGFTSESYQQGVLSATILYEILLGKATLYAVLVSALVLMAMVKRKDSRG

SEQ ID NO: 24 - protein, 311 aa, Homo sapiens
MDTWLVCWAIFSLLKAGLTEPEVTQTPSHQVTQMGQEVILRCVPISNHLYFYWYRQILGQKVEFLVSFYNNEISEKSEIFDDQFSVERPDGSNFTLKIRSTKLEDSAMYFCASSGQGANEQYFGPGTRLTVTEDLKNVFPPEVAVFEPSEAEISHTQKATLVCLATGFYPDHVELSWWVNGKEVHSGVSTDPQPLKEQPALNDSRYCLSSRLRVSATFWQNPRNHFRCQVQFYGLSENDEWTQDRAKPVTQIVSAEAWGRADCGFTSESYQQGVLSATILYEILLGKATLYAVLVSALVLMAMVKRKDSRG

SEQ ID NO: 25 - protein, 7 aa, Homo sapiens
TSESDYY

SEQ ID NO: 26 - protein, 4 aa, Homo sapiens
QEAY

SEQ ID NO: 27 - protein, 10 aa, Homo sapiens
CAYLNYQLIW

SEQ ID NO: 28 - protein, 131 aa, Homo sapiens
MACPGFLWALVISTCLEFSMAQTVTQSQPEMSVQEAETVTLSCTYDTSESDYYLFWYKQPPSRQMILVIRQEAYKQQNATENRFSVNFQKAAKSFSLKISDSQLGDAAMYFCAYLNYQLIWGAGTKLIIKP

SEQ ID NO: 29 - protein, 141 aa, Homo sapiens
DIQNPDPAVYQLRDSKSSDKSVCLFTDFDSQTNVSQSKDSDVYITDKTVLDMRSMDFKSNSAVAWSNKSDFACANAFNNSIIPEDTFFPSPESSCDVKLVEKSFETDTNLNFQNLSVIGFRILLLKVAGFNLLMTLRLWSS

SEQ ID NO: 30 - protein, 272 aa, Homo sapiens
MACPGFLWALVISTCLEFSMAQTVTQSQPEMSVQEAETVTLSCTYDTSESDYYLFWYKQPPSRQMILVIRQEAYKQQNATENRFSVNFQKAAKSFSLKISDSQLGDAAMYFCAYLNYQLIWGAGTKLIIKPDIQNPDPAVYQLRDSKSSDKSVCLFTDFDSQTNVSQSKDSDVYITDKTVLDMRSMDFKSNSAVAWSNKSDFACANAFNNSIIPEDTFFPSPESSCDVKLVEKSFETDTNLNFQNLSVIGFRILLLKVAGFNLLMTLRLWSS

SEQ ID NO: 31 - protein, 5 aa, Homo sapiens
SNHLY

SEQ ID NO: 32 - protein, 6 aa, Homo sapiens
FYNNEI

SEQ ID NO: 33 - protein, 13 aa, Homo sapiens
CASSEMTAVGQYF

SEQ ID NO: 34 - protein, 132 aa, Homo sapiens
MDTWLVCWAIFSLLKAGLTEPEVTQTPSHQVTQMGQEVILRCVPISNHLYFYWYRQILGQKVEFLVSFYNNEISEKSEIFDDQFSVERPDGSNFTLKIRSTKLEDSAMYFCASSEMTAVGQYFGPGTRLTVT

SEQ ID NO: 35 - protein, 179 aa, Homo sapiens; identical to SEQ ID NO: 23

SEQ ID NO: 36 - protein, 311 aa, Homo sapiens
MDTWLVCWAIFSLLKAGLTEPEVTQTPSHQVTQMGQEVILRCVPISNHLYFYWYRQILGQKVEFLVSFYNNEISEKSEIFDDQFSVERPDGSNFTLKIRSTKLEDSAMYFCASSEMTAVGQYFGPGTRLTVTEDLKNVFPPEVAVFEPSEAEISHTQKATLVCLATGFYPDHVELSWWVNGKEVHSGVSTDPQPLKEQPALNDSRYCLSSRLRVSATFWQNPRNHFRCQVQFYGLSENDEWTQDRAKPVTQIVSAEAWGRADCGFTSESYQQGVLSATILYEILLGKATLYAVLVSALVLMAMVKRKDSRG

SEQ ID NO: 37 - protein, 6 aa, Homo sapiens
DRGSQS

SEQ ID NO: 38 - protein, 2 aa, Homo sapiens
IY

SEQ ID NO: 39 - protein, 11 aa, Homo sapiens
CAAFSGYALNF

SEQ ID NO: 40 - protein, 130 aa, Homo sapiens
MKSLRVLLVILWLQLSWVWSQQKEVEQNSGPLSVPEGAIASLNCTYSDRGSQSFFWYRQYSGKSPELIMFIYSNGDKEDGRFTAQLNKASQYVSLLIRDSQPSDSATYLCAAFSGYALNFGKGTSLLVTP

SEQ ID NO: 41 - protein, 141 aa, Homo sapiens
HIQNPDPAVYQLRDSKSSDKSVCLFTDFDSQTNVSQSKDSDVYITDKTVLDMRSMDFKSNSAVAWSNKSDFACANAFNNSIIPEDTFFPSPESSCDVKLVEKSFETDTNLNFQNLSVIGFRILLLKVAGFNLLMTLRLWSS

SEQ ID NO: 42 - protein, 271 aa, Homo sapiens
MKSLRVLLVILWLQLSWVWSQQKEVEQNSGPLSVPEGAIASLNCTYSDRGSQSFFWYRQYSGKSPELIMFIYSNGDKEDGRFTAQLNKASQYVSLLIRDSQPSDSATYLCAAFSGYALNFGKGTSLLVTPHIQNPDPAVYQLRDSKSSDKSVCLFTDFDSQTNVSQSKDSDVYITDKTVLDMRSMDFKSNSAVAWSNKSDFACANAFNNSIIPEDTFFPSPESSCDVKLVEKSFETDTNLNFQNLSVIGFRILLLKVAGFNLLMTLRLWSS

SEQ ID NO: 43 - protein, 5 aa, Homo sapiens
SNHLY

SEQ ID NO: 44 - protein, 6 aa, Homo sapiens
FYNNEI

SEQ ID NO: 45 - protein, 12 aa, Homo sapiens
CASSQYTGELFF

SEQ ID NO: 46 - protein, 131 aa, Homo sapiens
MDTWLVCWAIFSLLKAGLTEPEVTQTPSHQVTQMGQEVILRCVPISNHLYFYWYRQILGQKVEFLVSFYNNEISEKSEIFDDQFSVERPDGSNFTLKIRSTKLEDSAMYFCASSQYTGELFFGEGSRLTVL

SEQ ID NO: 47 - protein, 179 aa, Homo sapiens; identical to SEQ ID NO: 23

SEQ ID NO: 48 - protein, 310 aa, Homo sapiens
MDTWLVCWAIFSLLKAGLTEPEVTQTPSHQVTQMGQEVILRCVPISNHLYFYWYRQILGQKVEFLVSFYNNEISEKSEIFDDQFSVERPDGSNFTLKIRSTKLEDSAMYFCASSQYTGELFFGEGSRLTVLEDLKNVFPPEVAVFEPSEAEISHTQKATLVCLATGFYPDHVELSWWVNGKEVHSGVSTDPQPLKEQPALNDSRYCLSSRLRVSATFWQNPRNHFRCQVQFYGLSENDEWTQDRAKPVTQIVSAEAWGRADCGFTSESYQQGVLSATILYEILLGKATLYAVLVSALVLMAMVKRKDSRG

SEQ ID NO: 49 - protein, 6 aa, Homo sapiens
DRGSQS

SEQ ID NO: 50 - protein, 2 aa, Homo sapiens
IY

SEQ ID NO: 51 - protein, 10 aa, Homo sapiens
CAVNGGDMRF

SEQ ID NO: 52 - protein, 129 aa, Homo sapiens
MKSLRVLLVILWLQLSWVWSQQKEVEQNSGPLSVPEGAIASLNCTYSDRGSQSFFWYRQYSGKSPELIMFIYSNGDKEDGRFTAQLNKASQYVSLLIRDSQPSDSATYLCAVNGGDMRFGAGTRLTVKP

SEQ ID NO: 53 - protein, 141 aa, Homo sapiens; identical to SEQ ID NO: 5

SEQ ID NO: 54 - protein, 270 aa, Homo sapiens
MKSLRVLLVILWLQLSWVWSQQKEVEQNSGPLSVPEGAIASLNCTYSDRGSQSFFWYRQYSGKSPELIMFIYSNGDKEDGRFTAQLNKASQYVSLLIRDSQPSDSATYLCAVNGGDMRFGAGTRLTVKPNIQNPDPAVYQLRDSKSSDKSVCLFTDFDSQTNVSQSKDSDVYITDKTVLDMRSMDFKSNSAVAWSNKSDFACANAFNNSIIPEDTFFPSPESSCDVKLVEKSFETDTNLNFQNLSVIGFRILLLKVAGFNLLMTLRLWSS

SEQ ID NO: 55 - protein, 5 aa, Homo sapiens
SNHLY

SEQ ID NO: 56 - protein, 6 aa, Homo sapiens
FYNNEI

SEQ ID NO: 57 - protein, 13 aa, Homo sapiens
CASSGQGALEQYF

SEQ ID NO: 58 - protein, 132 aa, Homo sapiens
MDTWLVCWAIFSLLKAGLTEPEVTQTPSHQVTQMGQEVILRCVPISNHLYFYWYRQILGQKVEFLVSFYNNEISEKSEIFDDQFSVERPDGSNFTLKIRSTKLEDSAMYFCASSGQGALEQYFGPGTRLTVT

SEQ ID NO: 59 - protein, 179 aa, Homo sapiens; identical to SEQ ID NO: 23

SEQ ID NO: 60 - protein, 311 aa, Homo sapiens
MDTWLVCWAIFSLLKAGLTEPEVTQTPSHQVTQMGQEVILRCVPISNHLYFYWYRQILGQKVEFLVSFYNNEISEKSEIFDDQFSVERPDGSNFTLKIRSTKLEDSAMYFCASSGQGALEQYFGPGTRLTVTEDLKNVFPPEVAVFEPSEAEISHTQKATLVCLATGFYPDHVELSWWVNGKEVHSGVSTDPQPLKEQPALNDSRYCLSSRLRVSATFWQNPRNHFRCQVQFYGLSENDEWTQDRAKPVTQIVSAEAWGRADCGFTSESYQQGVLSATILYEILLGKATLYAVLVSALVLMAMVKRKDSRG

SEQ ID NO: 61 - protein, 6 aa, Homo sapiens
NSMFDY

SEQ ID NO: 62 - protein, 3 aa, Homo sapiens
ISS

SEQ ID NO: 63 - protein, 15 aa, Homo sapiens
CAASGLYNQGGKLIF

SEQ ID NO: 64 - protein, 140 aa, Homo sapiens
MAMLLGASVLILWLQPDWVNSQQKNDDQQVKQNSPSLSVQEGRISILNCDYTNSMFDYFLWYKKYPAEGPTFLISISSIKDKNEDGRFTVFLNKSAKHLSLHIVPSQPGDSAVYFCAASGLYNQGGKLIFGQGTELSVKP

SEQ ID NO: 65 - protein, 141 aa, Homo sapiens; identical to SEQ ID NO: 5

SEQ ID NO: 66 - protein, 281 aa, Homo sapiens
MAMLLGASVLILWLQPDWVNSQQKNDDQQVKQNSPSLSVQEGRISILNCDYTNSMFDYFLWYKKYPAEGPTFLISISSIKDKNEDGRFTVFLNKSAKHLSLHIVPSQPGDSAVYFCAASGLYNQGGKLIFGQGTELSVKPNIQNPDPAVYQLRDSKSSDKSVCLFTDFDSQTNVSQSKDSDVYITDKTVLDMRSMDFKSNSAVAWSNKSDFACANAFNNSIIPEDTFFPSPESSCDVKLVEKSFETDTNLNFQNLSVIGFRILLLKVAGFNLLMTLRLWSS

SEQ ID NO: 67 - protein, 5 aa, Homo sapiens
LGHDT

SEQ ID NO: 68 - protein, 6 aa, Homo sapiens
YNNKEL

SEQ ID NO: 69 - protein, 14 aa, Homo sapiens
CASSLGDRGYEQYF

SEQ ID NO: 70 - protein, 132 aa, Homo sapiens
MGCRLLCCVVFCLLQAGPLDTAVSQTPKYLVTQMGNDKSIKCEQNLGHDTMYWYKQDSKKFLKIMFSYNNKELIINETVPNRFSPKSPDKAHLNLHINSLELGDSAVYFCASSLGDRGYEQYFGPGTRLTVT

SEQ ID NO: 71 - protein, 179 aa, Homo sapiens; identical to SEQ ID NO: 23

SEQ ID NO: 72 - protein, 311 aa, Homo sapiens
MGCRLLCCVVFCLLQAGPLDTAVSQTPKYLVTQMGNDKSIKCEQNLGHDTMYWYKQDSKKFLKIMFSYNNKELIINETVPNRFSPKSPDKAHLNLHINSLELGDSAVYFCASSLGDRGYEQYFGPGTRLTVTEDLKNVFPPEVAVFEPSEAEISHTQKATLVCLATGFYPDHVELSWWVNGKEVHSGVSTDPQPLKEQPALNDSRYCLSSRLRVSATFWQNPRNHFRCQVQFYGLSENDEWTQDRAKPVTQIVSAEAWGRADCGFTSESYQQGVLSATILYEILLGKATLYAVLVSALVLMAMVKRKDSRG

SEQ ID NO: 73 - protein, 6 aa, Homo sapiens
DSSSTY

SEQ ID NO: 74 - protein, 3 aa, Homo sapiens
IFS

SEQ ID NO: 75 - protein, 12 aa, Homo sapiens
CAEINNNARLMF

SEQ ID NO: 76 - protein, 131 aa, Homo sapiens
MKTFAGFSFLFLWLQLDCMSRGEDVEQSLFLSVREGDSSVINCTYTDSSSTYLYWYKQEPGAGLQLLTYIFSNMDMKQDQRLTVLLNKKDKHLSLRIADTQTGDSAIYFCAEINNNARLMFGDGTQLVVKP

SEQ ID NO: 77 - protein, 141 aa, Homo sapiens; identical to SEQ ID NO: 5

SEQ ID NO: 78 - protein, 272 aa, Homo sapiens
MKTFAGFSFLFLWLQLDCMSRGEDVEQSLFLSVREGDSSVINCTYTDSSSTYLYWYKQEPGAGLQLLTYIFSNMDMKQDQRLTVLLNKKDKHLSLRIADTQTGDSAIYFCAEINNNARLMFGDGTQLVVKPNIQNPDPAVYQLRDSKSSDKSVCLFTDFDSQTNVSQSKDSDVYITDKTVLDMRSMDFKSNSAVAWSNKSDFACANAFNNSIIPEDTFFPSPESSCDVKLVEKSFETDTNLNFQNLSVIGFRILLLKVAGFNLLMTLRLWSS

SEQ ID NO: 79 - protein, 5 aa, Homo sapiens
PRHDT

SEQ ID NO: 80 - protein, 6 aa, Homo sapiens
FYEKMQ

SEQ ID NO: 81 - protein, 13 aa, Homo sapiens
CASSPPDQNTQYF

SEQ ID NO: 82 - protein, 141 aa, Homo sapiens
MLSPDLPDSAWNTRLLCHVMLCLLGAVSVAAGVIQSPRHLIKEKRETATLKCYPIPRHDTVYWYQQGPGQDPQFLISFYEKMQSDKGSIPDRFSAQQFSDYHSELNMSSLELGDSALYFCASSPPDQNTQYFGPGTRLTVL

SEQ ID NO: 83 - protein, 179 aa, Homo sapiens; identical to SEQ ID NO: 23

SEQ ID NO: 84 - protein, 320 aa, Homo sapiens
MLSPDLPDSAWNTRLLCHVMLCLLGAVSVAAGVIQSPRHLIKEKRETATLKCYPIPRHDTVYWYQQGPGQDPQFLISFYEKMQSDKGSIPDRFSAQQFSDYHSELNMSSLELGDSALYFCASSPPDQNTQYFGPGTRLTVLEDLKNVFPPEVAVFEPSEAEISHTQKATLVCLATGFYPDHVELSWWVNGKEVHSGVSTDPQPLKEQPALNDSRYCLSSRLRVSATFWQNPRNHFRCQVQFYGLSENDEWTQDRAKPVTQIVSAEAWGRADCGFTSESYQQGVLSATILYEILLGKATLYAVLVSALVLMAMVKRKDSRG

SEQ ID NO: 85 - protein, 6 aa, Homo sapiens
SSVPPY

SEQ ID NO: 86 - protein, 4 aa, Homo sapiens
YTTG

SEQ ID NO: 87 - protein, 13 aa, Homo sapiens
CAVRIFGNEKLTF

SEQ ID NO: 88 - protein, 132 aa, Homo sapiens
MLLLLVPVLEVIFTLGGTRAQSVTQLGSHVSVSEGALVLLRCNYSSSVPPYLFWYVQYPNQGLQLLLKYTTGATLVKGINGFEAEFKKSETSFHLTKPSAHMSDAAEYFCAVRIFGNEKLTFGTGTRLTIIP

SEQ ID NO: 89 - protein, 141 aa, Homo sapiens; identical to SEQ ID NO: 5

SEQ ID NO: 90 - protein, 273 aa, Homo sapiens
MLLLLVPVLEVIFTLGGTRAQSVTQLGSHVSVSEGALVLLRCNYSSSVPPYLFWYVQYPNQGLQLLLKYTTGATLVKGINGFEAEFKKSETSFHLTKPSAHMSDAAEYFCAVRIFGNEKLTFGTGTRLTIIPNIQNPDPAVYQLRDSKSSDKSVCLFTDFDSQTNVSQSKDSDVYITDKTVLDMRSMDFKSNSAVAWSNKSDFACANAFNNSIIPEDTFFPSPESSCDVKLVEKSFETDTNLNFQNLSVIGFRILLLKVAGFNLLMTLRLWSS

SEQ ID NO: 91 - protein, 5 aa, Homo sapiens
MDHEN

SEQ ID NO: 92 - protein, 6 aa, Homo sapiens
SYDVKM

SEQ ID NO: 93 - protein, 15 aa, Homo sapiens
CASSLMGELTGELFF

SEQ ID NO: 94 - protein, 133 aa, Homo sapiens
MGIRLLCRVAFCFLAVGLVDVKVTQSSRYLVKRTGEKVFLECVQDMDHENMFWYRQDPGLGLRLIYFSYDVKMKEKGDIPEGYSVSREKKERFSLILESASTNQTSMYLCASSLMGELTGELFFGEGSRLTVL

SEQ ID NO: 95 - protein, 179 aa, Homo sapiens; identical to SEQ ID NO: 23

SEQ ID NO: 96 - protein, 312 aa, Homo sapiens
MGIRLLCRVAFCFLAVGLVDVKVTQSSRYLVKRTGEKVFLECVQDMDHENMFWYRQDPGLGLRLIYFSYDVKMKEKGDIPEGYSVSREKKERFSLILESASTNQTSMYLCASSLMGELTGELFFGEGSRLTVLEDLKNVFPPEVAVFEPSEAEISHTQKATLVCLATGFYPDHVELSWWVNGKEVHSGVSTDPQPLKEQPALNDSRYCLSSRLRVSATFWQNPRNHFRCQVQFYGLSENDEWTQDRAKPVTQIVSAEAWGRADCGFTSESYQQGVLSATILYEILLGKATLYAVLVSALVLMAMVKRKDSRG

SEQ ID NO: 97 - protein, 6 aa, Homo sapiens
NSAFQY

SEQ ID NO: 98 - protein, 2 aa, Homo sapiens
TY

SEQ ID NO: 99 - protein, 15 aa, Homo sapiens
CAMMGDTGTASKLTF

SEQ ID NO: 100 - protein, 135 aa, Homo sapiens
MMKSLRVLLVILWLQLSWVWSQQKEVEQDPGPLSVPEGAIVSLNCTYSNSAFQYFMWYRQYSRKGPELLMYTYSSGNKEDGRFTAQVDKSSKYISLFIRDSQPSDSATYLCAMMGDTGTASKLTFGTGTRLQVTL

SEQ ID NO: 101 - protein, 141 aa, Homo sapiens; identical to SEQ ID NO: 29

SEQ ID NO: 102 - protein, 276 aa, Homo sapiens
MMKSLRVLLVILWLQLSWVWSQQKEVEQDPGPLSVPEGAIVSLNCTYSNSAFQYFMWYRQYSRKGPELLMYTYSSGNKEDGRFTAQVDKSSKYISLFIRDSQPSDSATYLCAMMGDTGTASKLTFGTGTRLQVTLDIQNPDPAVYQLRDSKSSDKSVCLFTDFDSQTNVSQSKDSDVYITDKTVLDMRSMDFKSNSAVAWSNKSDFACANAFNNSIIPEDTFFPSPESSCDVKLVEKSFETDTNLNFQNLSVIGFRILLLKVAGFNLLMTLRLWSS

SEQ ID NO: 103 - protein, 5 aa, Homo sapiens
MDHEN

SEQ ID NO: 104 - protein, 6 aa, Homo sapiens
SYDVKM

SEQ ID NO: 105 - protein, 12 aa, Homo sapiens
CASSFGGYEQYF

SEQ ID NO: 106 - protein, 130 aa, Homo sapiens
MGIRLLCRVAFCFLAVGLVDVKVTQSSRYLVKRTGEKVFLECVQDMDHENMFWYRQDPGLGLRLIYFSYDVKMKEKGDIPEGYSVSREKKERFSLILESASTNQTSMYLCASSFGGYEQYFGPGTRLTVT

SEQ ID NO: 107 - protein, 179 aa, Homo sapiens; identical to SEQ ID NO: 23

SEQ ID NO: 108 - protein, 309 aa, Homo sapiens
MGIRLLCRVAFCFLAVGLVDVKVTQSSRYLVKRTGEKVFLECVQDMDHENMFWYRQDPGLGLRLIYFSYDVKMKEKGDIPEGYSVSREKKERFSLILESASTNQTSMYLCASSFGGYEQYFGPGTRLTVTEDLKNVFPPEVAVFEPSEAEISHTQKATLVCLATGFYPDHVELSWWVNGKEVHSGVSTDPQPLKEQPALNDSRYCLSSRLRVSATFWQNPRNHFRCQVQFYGLSENDEWTQDRAKPVTQIVSAEAWGRADCGFTSESYQQGVLSATILYEILLGKATLYAVLVSALVLMAMVKRKDSRG

SEQ ID NO: 109 - protein, 6 aa, Homo sapiens
DRGSQS

SEQ ID NO: 110 - protein, 2 aa, Homo sapiens
IY

SEQ ID NO: 111 - protein, 10 aa, Homo sapiens
CAVQPHDMRF

SEQ ID NO: 112 - protein, 129 aa, Homo sapiens
MKSLRVLLVILWLQLSWVWSQQKEVEQNSGPLSVPEGAIASLNCTYSDRGSQSFFWYRQYSGKSPELIMSIYSNGDKEDGRFTAQLNKASQYVSLLIRDSQPSDSATYLCAVQPHDMRFGAGTRLTVKP

SEQ ID NO: 113 - protein, 141 aa, Homo sapiens; identical to SEQ ID NO: 5

SEQ ID NO: 114 - protein, 270 aa, Homo sapiens
MKSLRVLLVILWLQLSWVWSQQKEVEQNSGPLSVPEGAIASLNCTYSDRGSQSFFWYRQYSGKSPELIMSIYSNGDKEDGRFTAQLNKASQYVSLLIRDSQPSDSATYLCAVQPHDMRFGAGTRLTVKPNIQNPDPAVYQLRDSKSSDKSVCLFTDFDSQTNVSQSKDSDVYITDKTVLDMRSMDFKSNSAVAWSNKSDFACANAFNNSIIPEDTFFPSPESSCDVKLVEKSFETDTNLNFQNLSVIGFRILLLKVAGFNLLMTLRLWSS

SEQ ID NO: 115 - protein, 6 aa, Homo sapiens
GTSNPN

SEQ ID NO: 116 - protein, 5 aa, Homo sapiens
SVGIG

SEQ ID NO: 117 - protein, 12 aa, Homo sapiens
CAWSGLVAEQFF

SEQ ID NO: 118 - protein, 128 aa, Homo sapiens
MLCSLLALLLGTFFGVRSQTIHQWPATLVQPVGSPLSLECTVEGTSNPNLYWYRQAAGRGLQLLFYSVGIGQISSEVPQNLSASRPQDRQFILSSKKLLLSDSGFYLCAWSGLVAEQFFGPGTRLTVL

SEQ ID NO: 119 - protein, 179 aa, Homo sapiens; identical to SEQ ID NO: 23

SEQ ID NO: 120 - protein, 307 aa, Homo sapiens
MLCSLLALLLGTFFGVRSQTIHQWPATLVQPVGSPLSLECTVEGTSNPNLYWYRQAAGRGLQLLFYSVGIGQISSEVPQNLSASRPQDRQFILSSKKLLLSDSGFYLCAWSGLVAEQFFGPGTRLTVLEDLKNVFPPEVAVFEPSEAEISHTQKATLVCLATGFYPDHVELSWWVNGKEVHSGVSTDPQPLKEQPALNDSRYCLSSRLRVSATFWQNPRNHFRCQVQFYGLSENDEWTQDRAKPVTQIVSAEAWGRADCGFTSESYQQGVLSATILYEILLGKATLYAVLVSALVLMAMVKRKDSRG

SEQ ID NO: 121 - protein, 6 aa, Homo sapiens
DSAIYN

SEQ ID NO: 122 - protein, 3 aa, Homo sapiens
IQS

SEQ ID NO: 123 - protein, 15 aa, Homo sapiens
CAVRPTSGGSYIPTF

SEQ ID NO: 124 - protein, 133 aa, Homo sapiens
METLLGLLILWLQLQWVSSKQEVTQIPAALSVPEGENLVLNCSFTDSAIYNLQWFRQDPGKGLTSLLLIQSSQREQTSGRLNASLDKSSGRSTLYIAASQPGDSATYLCAVRPTSGGSYIPTFGRGTSLIVHP

SEQ ID NO: 125 - protein, 141 aa, Homo sapiens
YIQNPDPAVYQLRDSKSSDKSVCLFTDFDSQTNVSQSKDSDVYITDKTVLDMRSMDFKSNSAVAWSNKSDFACANAFNNSIIPEDTFFPSPESSCDVKLVEKSFETDTNLNFQNLSVIGFRILLLKVAGFNLLMTLRLWSS

SEQ ID NO: 126 - protein, 274 aa, Homo sapiens
METLLGLLILWLQLQWVSSKQEVTQIPAALSVPEGENLVLNCSFTDSAIYNLQWFRQDPGKGLTSLLLIQSSQREQTSGRLNASLDKSSGRSTLYIAASQPGDSATYLCAVRPTSGGSYIPTFGRGTSLIVHPYIQNPDPAVYQLRDSKSSDKSVCLFTDFDSQTNVSQSKDSDVYITDKTVLDMRSMDFKSNSAVAWSNKSDFACANAFNNSIIPEDTFFPSPESSCDVKLVEKSFETDTNLNFQNLSVIGFRILLLKVAGFNLLMTLRLWSS

SEQ ID NO: 127 - protein, 5 aa, Homo sapiens
MNHEY

SEQ ID NO: 128 - protein, 6 aa, Homo sapiens
SVGAGI

SEQ ID NO: 129 - protein, 14 aa, Homo sapiens
CASSYVGNTGELFF

SEQ ID NO: 130 - protein, 132 aa, Homo sapiens
MSIGLLCCAALSLLWAGPVNAGVTQTPKFQVLKTGQSMTLQCAQDMNHEYMSWYRQDPGMGLRLIHYSVGAGITDQGEVPNGYNVSRSTTEDFPLRLLSAAPSQTSVYFCASSYVGNTGELFFGEGSRLTVL

SEQ ID NO: 131 - protein, 179 aa, Homo sapiens; identical to SEQ ID NO: 23

SEQ ID NO: 132 - protein, 311 aa, Homo sapiens
MSIGLLCCAALSLLWAGPVNAGVTQTPKFQVLKTGQSMTLQCAQDMNHEYMSWYRQDPGMGLRLIHYSVGAGITDQGEVPNGYNVSRSTTEDFPLRLLSAAPSQTSVYFCASSYVGNTGELFFGEGSRLTVLEDLKNVFPPEVAVFEPSEAEISHTQKATLVCLATGFYPDHVELSWWVNGKEVHSGVSTDPQPLKEQPALNDSRYCLSSRLRVSATFWQNPRNHFRCQVQFYGLSENDEWTQDRAKPVTQIVSAEAWGRADCGFTSESYQQGVLSATILYEILLGKATLYAVLVSALVLMAMVKRKDSRG

SEQ ID NO: 133 - protein, 9 aa, Homo sapiens
ALSVLRLAL

SEQ ID NO: 134 - protein, 9 aa, Homo sapiens
AASVLRLAL

SEQ ID NO: 135 - protein, 9 aa, Homo sapiens
ALAVLRLAL

SEQ ID NO: 136 - protein, 9 aa, Homo sapiens
ALSALRLAL

SEQ ID NO: 137 - protein, 9 aa, Homo sapiens
ALSVARLAL

SEQ ID NO: 138 - protein, 9 aa, Homo sapiens
ALSVLALAL

SEQ ID NO: 139 - protein, 9 aa, Homo sapiens
ALSVLRAAL

SEQ ID NO: 140 - protein, 9 aa, Homo sapiens
ALSVLRLAA

SEQ ID NO: 141 - protein, 9 aa, Homo sapiens
TLSVLRLAL

SEQ ID NO: 142 - protein, 9 aa, Homo sapiens
ATSVLRLAL

SEQ ID NO: 143 - protein, 9 aa, Homo sapiens
ALTVLRLAL

SEQ ID NO: 144 - protein, 9 aa, Homo sapiens
ALSTLRLAL

SEQ ID NO: 145 - protein, 9 aa, Homo sapiens
ALSVTRLAL

SEQ ID NO: 146 - protein, 9 aa, Homo sapiens
ALSVLTLAL

SEQ ID NO: 147 - protein, 9 aa, Homo sapiens
ALSVLRTAL

SEQ ID NO: 148 - protein, 9 aa, Homo sapiens
ALSVLRLTL

SEQ ID NO: 149 - protein, 9 aa, Homo sapiens
ALSVLRLAT

SEQ ID NO: 150 - protein, 9 aa, Homo sapiens
ALMNMKLAL

SEQ ID NO: 151 - protein, 9 aa, Homo sapiens
ALSDLRCNL

SEQ ID NO: 152 - protein, 9 aa, Homo sapiens
ALSSLIHAL

SEQ ID NO: 153 - protein, 9 aa, Homo sapiens
ALSTLALYV

SEQ ID NO: 154 - protein, 9 aa, Homo sapiens
ALSVLADFL

SEQ ID NO: 155 - protein, 9 aa, Homo sapiens
ALYASRLYL

SEQ ID NO: 156 - protein, 9 aa, Homo sapiens
GLSDLRLEL

SEQ ID NO: 157 - protein, 9 aa, Homo sapiens
IVSSLRLAY

SEQ ID NO: 158 - protein, 9 aa, Homo sapiens
YLDVIRLLL

SEQ ID NO: 159 - protein, 9 aa, Homo sapiens
SLLMWITQV